European Patent Application EP 4 115 909 A1, published January 11, 2023. Title: ANTIBODY-DRUG CONJUGATE CONTAINING NOVEL CYCLIC DINUCLEOTIDE DERIVATIVE. Applicant: DAIICHI SANKYO COMPANY, LIMITED. The sequence listing filed with the application follows.

SEQUENCE LISTING (70 sequences)

SEQ ID NO: 1 - protein, 218 aa, Homo sapiens
DIVMTQSPDSLAVSLGERATINCRASKSVSTSGYSFMHWYQQKPGQPPKLLIYLASNLESGVPDRFSGSGSGTDFTLTISSLQAEDVAVYYCQHSREVPWTFGQGTKVEIKRTVAAPSVFIFPPSDEQLKSGTASVVCLLNNFYPREAKVQWKVDNALQSGNSQESVTEQDSKDSTYSLSSTLTLSKADYEKHKVYACEVTHQGLSSPVTKSFNRGEC

SEQ ID NO: 2 - protein, 448 aa, Homo sapiens
QVQLVQSGAEVKKPGASVKVSCKASGYTFTNYGMNWVRQAPGQGLKWMGWINTYTGEPTYADAFKGRVTMTRDTSISTAYMELSRLRSDDTAVYYCARDYGDYGMDYWGQGTTVTVSSASTKGPSVFPLAPSSKSTSGGTAALGCLVKDYFPEPVTVSWNSGALTSGVHTFPAVLQSSGLYSLSSVVTVPSSSLGTQTYICNVNHKPSNTKVDKRVEPKSCDKTHTCPPCPAPEAAGGPSVFLFPPKPKDTLMISRTPEVTCVVVDVSHEDPEVKFNWYVDGVEVHNAKTKPREEQYNSTYRVVSVLTVLHQDWLNGKEYKCKVSNKALPAPIEKTISKAKGQPREPQVYTLPPSREEMTKNQVSLTCLVKGFYPSDIAVEWESNGQPENNYKTTPPVLDSDGSFFLYSKLTVDKSRWQQGNVFSCSVMHEALHNHYTQKSLSLSPGK

SEQ ID NO: 3 - protein, 214 aa, Homo sapiens
EIVLTQSPATLSLSPGERATLSCRASQSVSSYLAWYQQKPGQAPRLLIYDASNRATGIPARFSGSGSGTDFTLTISSLEPEDFAVYYCQQRTNWPLTFGGGTKVEIKRTVAAPSVFIFPPSDEQLKSGTASVVCLLNNFYPREAKVQWKVDNALQSGNSQESVTEQDSKDSTYSLSSTLTLSKADYEKHKVYACEVTHQGLSSPVTKSFNRGEC

SEQ ID NO: 4 - protein, 448 aa, Homo sapiens
QVQLVESGGGVVQPGRSLRLSCAASGFTFSSYIMHWVRQAPGKGLEWVAVISYDGRNKYYADSVKGRFTISRDNSKNTLYLQMNSLRAEDTAVYYCARDTDGYDFDYWGQGTLVTVSSASTKGPSVFPLAPSSKSTSGGTAALGCLVKDYFPEPVTVSWNSGALTSGVHTFPAVLQSSGLYSLSSVVTVPSSSLGTQTYICNVNHKPSNTKVDKRVEPKSCDKTHTCPPCPAPEAAGGPSVFLFPPKPKDTLMISRTPEVTCVVVDVSHEDPEVKFNWYVDGVEVHNAKTKPREEQYNSTYRVVSVLTVLHQDWLNGKEYKCKVSNKALPAPIEKTISKAKGQPREPQVYTLPPSREEMTKNQVSLTCLVKGFYPSDIAVEWESNGQPENNYKTTPPVLDSDGSFFLYSKLTVDKSRWQQGNVFSCSVMHEALHNHYTQKSLSLSPGK

SEQ ID NO: 5 - protein, 214 aa, Homo sapiens
DIQMTQSPSSLSASVGDRVTITCKASQDVSTAVAWYQQKPGKAPKLLIYSASYRYTGVPSRFSGSGSGTDFTLTISSLQPEDFAVYYCQQHYITPLTFGQGTKLEIKRTVAAPSVFIFPPSDEQLKSGTASVVCLLNNFYPREAKVQWKVDNALQSGNSQESVTEQDSKDSTYSLSSTLTLSKADYEKHKVYACEVTHQGLSSPVTKSFNRGEC

SEQ ID NO: 6 - protein, 451 aa, Homo sapiens
QVQLVQSGAEVKKPGASVKVSCKASGYTFTTAGMQWVRQAPGQGLEWMGWINTHSGVPKYAEDFKGRVTISADTSTSTAYLQLSSLKSEDTAVYYCARSGFGSSYWYFDVWGQGTLVTVSSASTKGPSVFPLAPSSKSTSGGTAALGCLVKDYFPEPVTVSWNSGALTSGVHTFPAVLQSSGLYSLSSVVTVPSSSLGTQTYICNVNHKPSNTKVDKRVEPKSCDKTHTCPPCPAPELLGGPSVFLFPPKPKDTLMISRTPEVTCVVVDVSHEDPEVKFNWYVDGVEVHNAKTKPREEQYNSTYRVVSVLTVLHQDWLNGKEYKCKVSNKALPAPIEKTISKAKGQPREPQVYTLPPSREEMTKNQVSLTCLVKGFYPSDIAVEWESNGQPENNYKTTPPVLDSDGSFFLYSKLTVDKSRWQQGNVFSCSVMHEALHNHYTQKSLSLSPGK

SEQ ID NO: 7 - protein, 214 aa, Homo sapiens; identical to SEQ ID NO: 5

SEQ ID NO: 8 - protein, 451 aa, Homo sapiens
QVQLVQSGAEVKKPGASVKVSCKASGYTFTTAGMQWVRQAPGQGLEWMGWINTHSGVPKYAEDFKGRVTISADTSTSTAYLQLSSLKSEDTAVYYCARSGFGSSYWYFDVWGQGTLVTVSSASTKGPSVFPLAPSSKSTSGGTAALGCLVKDYFPEPVTVSWNSGALTSGVHTFPAVLQSSGLYSLSSVVTVPSSSLGTQTYICNVNHKPSNTKVDKRVEPKSCDKTHTCPPCPAPEAAGGPSVFLFPPKPKDTLMISRTPEVTCVVVDVSHEDPEVKFNWYVDGVEVHNAKTKPREEQYNSTYRVVSVLTVLHQDWLNGKEYKCKVSNKALPAPIEKTISKAKGQPREPQVYTLPPSREEMTKNQVSLTCLVKGFYPSDIAVEWESNGQPENNYKTTPPVLDSDGSFFLYSKLTVDKSRWQQGNVFSCSVMHEALHNHYTQKSLSLSPGK

SEQ ID NO: 9 - protein, 214 aa, Homo sapiens
DIQMTQSPSSLSASVGDRVTITCQASQDISNYLNWYQQKPGKAPKLLIYDASNLETGVPSRFSGSGSGTDFTFTISSLQPEDIATYFCQHFDHLPLAFGGGTKVEIKRTVAAPSVFIFPPSDEQLKSGTASVVCLLNNFYPREAKVQWKVDNALQSGNSQESVTEQDSKDSTYSLSSTLTLSKADYEKHKVYACEVTHQGLSSPVTKSFNRGEC

SEQ ID NO: 10 - protein, 449 aa, Homo sapiens
QVQLQESGPGLVKPSETLSLTCTVSGGSVSSGDYYWTWIRQSPGKGLEWIGHIYYSGNTNYNPSLKSRLTISIDTSKTQFSLKLSSVTAADTAIYYCVRDRVTGAFDIWGQGTMVTVSSASTKGPSVFPLAPSSKSTSGGTAALGCLVKDYFPEPVTVSWNSGALTSGVHTFPAVLQSSGLYSLSSVVTVPSSSLGTQTYICNVNHKPSNTKVDKRVEPKSCDKTHTCPPCPAPEAAGGPSVFLFPPKPKDTLMISRTPEVTCVVVDVSHEDPEVKFNWYVDGVEVHNAKTKPREEQYNSTYRVVSVLTVLHQDWLNGKEYKCKVSNKALPAPIEKTISKAKGQPREPQVYTLPPSREEMTKNQVSLTCLVKGFYPSDIAVEWESNGQPENNYKTTPPVLDSDGSFFLYSKLTVDKSRWQQGNVFSCSVMHEALHNHYTQKSLSLSPGK

SEQ ID NO: 11 - protein, 214 aa, Homo sapiens
DILMTQSPSSMSVSLGDTVSITCHSSQDINSNIGWLQQRPGKSFKGLIYHGTNLDDEVPSRFSGSGSGADYSLTISSLESEDFADYYCVQYAQFPWTFGGGTKLEIKRTVAAPSVFIFPPSDEQLKSGTASVVCLLNNFYPREAKVQWKVDNALQSGNSQESVTEQDSKDSTYSLSSTLTLSKADYEKHKVYACEVTHQGLSSPVTKSFNRGEC

SEQ ID NO: 12 - protein, 446 aa, Homo sapiens
DVQLQESGPSLVKPSQSLSLTCTVTGYSITSDFAWNWIRQFPGNKLEWMGYISYSGNTRYNPSLKSRISITRDTSKNQFFLQLNSVTIEDTATYYCVTAGRGFPYWGQGTLVTVSAASTKGPSVFPLAPSSKSTSGGTAALGCLVKDYFPEPVTVSWNSGALTSGVHTFPAVLQSSGLYSLSSVVTVPSSSLGTQTYICNVNHKPSNTKVDKRVEPKSCDKTHTCPPCPAPEAAGGPSVFLFPPKPKDTLMISRTPEVTCVVVDVSHEDPEVKFNWYVDGVEVHNAKTKPREEQYNSTYRVVSVLTVLHQDWLNGKEYKCKVSNKALPAPIEKTISKAKGQPREPQVYTLPPSREEMTKNQVSLTCLVKGFYPSDIAVEWESNGQPENNYKTTPPVLDSDGSFFLYSKLTVDKSRWQQGNVFSCSVMHEALHNHYTQKSLSLSPGK

SEQ ID NO: 13 - protein, 379 aa, Homo sapiens [sequence omitted]

SEQ ID NO: 14 - DNA, 1140 bp, Homo sapiens
atgccccactccagcctgcatccatccatcccgtgtcccaggggtcacggggcccagaaggcagccttggttctgctgagtgcctgcctggtgaccctttgggggctaggagagccaccagagcacactctccggtacctggtgctccacctagcctccctgcagctgggactgctgttaaacggggtctgcagcctggctgaggagctgcgccacatccactccaggtaccggggcagctactggaggactgtgcgggcctgcctgggctgccccctccgccgtggggccctgttgctgctgtccatctatttctactactccctcccaaatgcggtcggcccgcccttcacttggatgcttgccctcctgggcctctcgcaggcactgaacatcctcctgggcctcaagggcctggccccagctgagatctctgcagtgtgtgaaaaagggaatttcaacgtggcccatgggctggcatggtcatattacatcggatatctgcggctgatcctgccagagctccaggcccggattcgaacttacaatcagcattacaacaacctgctacggggtgcagtgagccagcggctgtatattctcctcccattggactgtggggtgcctgataacctgagtatggctgaccccaacattcgcttcctggataaactgccccagcagaccggtgaccatgctggcatcaaggatcgggtttacagcaacagcatctatgagcttctggagaacgggcagcgggcgggcacctgtgtcctggagtacgccacccccttgcagactttgtttgccatgtcacaatacagtcaagctggctttagccgggaggataggcttgagcaggccaaactcttctgccggacacttgaggacatcctggcagatgcccctgagtctcagaacaactgccgcctcattgcctaccaggaacctgcagatgacagcagcttctcgctgtcccaggaggttctccggcacctgcggcaggaggaaaaggaagaggttactgtgggcagcttgaagacctcagcggtgcccagtacctccacgatgtcccaagagcctgagctcctcatcagtggaatggaaaagcccctccctctccgcacggatttctcttag

SEQ ID NO: 15 - protein, 379 aa, Homo sapiens
MPHSSLHPSIPCPRGHGAQKAALVLLSACLVTLWGLGEPPEHTLRYLVLHLASLQLGLLLNGVCSLAEELRHIHSRYRGSYWRTVRACLGCPLRRGALLLLSIYFYYSLPNAVGPPFTWMLALLGLSQALNILLGLKGLAPAEISAVCEKGNFNVAHGLAWSYYIGYLRLILPELQARIRTYNQHYNNLLRGAVSQRLYILLPLDCGVPDNLSMADPNIRFLDKLPQQTGDHAGIKDRVYSNSIYELLENGQRAGTCVLEYATPLQTLFAMSQYSQAGFSREDRLEQAKLFCRTLEDILADAPESQNNCRLIAYQEPADDSSFSLSQEVLRHLRQEEKEEVTVGSLKTSAVPSTSTMSQEPELLISGMEKPLPLRTDFS

SEQ ID NO: 16 - DNA, 1140 bp, Homo sapiens
atgccccactccagcctgcatccatccatcccgtgtcccaggggtcacggggcccagaaggcagccttggttctgctgagtgcctgcctggtgaccctttgggggctaggagagccaccagagcacactctccggtacctggtgctccacctagcctccctgcagctgggactgctgttaaacggggtctgcagcctggctgaggagctgcgccacatccactccaggtaccggggcagctactggaggactgtgcgggcctgcctgggctgccccctccgccgtggggccctgttgctgctgtccatctatttctactactccctcccaaatgcggtcggcccgcccttcacttggatgcttgccctcctgggcctctcgcaggcactgaacatcctcctgggcctcaagggcctggccccagctgagatctctgcagtgtgtgaaaaagggaatttcaacgtggcccatgggctggcatggtcatattacatcggatatctgcggctgatcctgccagagctccaggcccggattcgaacttacaatcagcattacaacaacctgctacggggtgcagtgagccagcggctgtatattctcctcccattggactgtggggtgcctgataacctgagtatggctgaccccaacattcgcttcctggataaactgccccagcagaccggtgaccgtgctggcatcaaggatcgggtttacagcaacagcatctatgagcttctggagaacgggcagcgggcgggcacctgtgtcctggagtacgccacccccttgcagactttgtttgccatgtcacaatacagtcaagctggctttagccgggaggataggcttgagcaggccaaactcttctgccggacacttgaggacatcctggcagatgcccctgagtctcagaacaactgccgcctcattgcctaccaggaacctgcagatgacagcagcttctcgctgtcccaggaggttctccggcacctgcggcaggaggaaaaggaagaggttactgtgggcagcttgaagacctcagcggtgcccagtacctccacgatgtcccaagagcctgagctcctcatcagtggaatggaaaagcccctccctctccgcacggatttctcttag

SEQ ID NO: 17 - protein, 379 aa, Homo sapiens
MPHSSLHPSIPCPRGHGAQKAALVLLSACLVTLWGLGEPPEHTLRYLVLHLASLQLGLLLNGVCSLAEELHHIHSRYRGSYWRTVRACLGCPLRRGALLLLSIYFYYSLPNAVGPPFTWMLALLGLSQALNILLGLKGLAPAEISAVCEKGNFNVAHGLAWSYYIGYLRLILPELQARIRTYNQHYNNLLRGAVSQRLYILLPLDCGVPDNLSMADPNIRFLDKLPQQTADRAGIKDRVYSNSIYELLENGQRAGTCVLEYATPLQTLFAMSQYSQAGFSREDRLEQAKLFCQTLEDILADAPESQNNCRLIAYQEPADDSSFSLSQEVLRHLRQEEKEEVTVGSLKTSAVPSTSTMSQEPELLISGMEKPLPLRTDFS

SEQ ID NO: 18 - DNA, 1140 bp, Homo sapiens
atgccccactccagcctgcatccatccatcccgtgtcccaggggtcacggggcccagaaggcagccttggttctgctgagtgcctgcctggtgaccctttgggggctaggagagccaccagagcacactctccggtacctggtgctccacctagcctccctgcagctgggactgctgttaaacggggtctgcagcctggctgaggagctgcaccacatccactccaggtaccggggcagctactggaggactgtgcgggcctgcctgggctgccccctccgccgtggggccctgttgctgctgtccatctatttctactactccctcccaaatgcggtcggcccgcccttcacttggatgcttgccctcctgggcctctcgcaggcactgaacatcctcctgggcctcaagggcctggccccagctgagatctctgcagtgtgtgaaaaagggaatttcaacgtggcccatgggctggcatggtcatattacatcggatatctgcggctgatcctgccagagctccaggcccggattcgaacttacaatcagcattacaacaacctgctacggggtgcagtgagccagcggctgtatattctcctcccattggactgtggggtgcctgataacctgagtatggctgaccccaacattcgcttcctggataaactgccccagcagaccgctgaccgtgctggcatcaaggatcgggtttacagcaacagcatctatgagcttctggagaacgggcagcgggcgggcacctgtgtcctggagtacgccacccccttgcagactttgtttgccatgtcacaatacagtcaagctggctttagccgggaggataggcttgagcaggccaaactcttctgccagacacttgaggacatcctggcagatgcccctgagtctcagaacaactgccgcctcattgcctaccaggaacctgcagatgacagcagcttctcgctgtcccaggaggttctccggcacctgcggcaggaggaaaaggaagaggttactgtgggcagcttgaagacctcagcggtgcccagtacctccacgatgtcccaagagcctgagctcctcatcagtggaatggaaaagcccctccctctccgcacggatttctcttag

SEQ ID NO: 19 - protein, 378 aa, Mus musculus
MPYSNLHPAIPRPRGHRSKYVALIFLVASLMILWVAKDPPNHTLKYLALHLASHELGLLLKNLCCLAEELCHVQSRYQGSYWKAVRACLGCPIHCMAMILLSSYFYFLQNTADIYLSWMFGLLVLYKSLSMLLGLQSLTPAEVSAVCEEKKLNVAHGLAWSYYIGYLRLILPGLQARIRMFNQLHNNMLSGAGSRRLYILFPLDCGVPDNLSVVDPNIRFRDMLPQQNIDRAGIKNRVYSNSVYEILENGQPAGVCILEYATPLQTLFAMSQDAKAGFSREDRLEQAKLFCRTLEEILEDVPESRNNCRLIVYQEPTDGNSFSLSQEVLRHIRQEEKEEVTMNAPMTSVAPPPSVLSQEPRLLISGMDQPLPLRTDLI

SEQ ID NO: 20 - DNA, 1137 bp, Mus musculus
atgccatactccaacctgcatccagccatcccacggcccagaggtcaccgctccaaatatgtagccctcatctttctggtggccagcctgatgatcctttgggtggcaaaggatccaccaaatcacactctgaagtacctagcacttcacctagcctcgcacgaacttggactactgttgaaaaacctctgctgtctggctgaagagctgtgccatgtccagtccaggtaccagggcagctactggaaggctgtgcgcgcctgcctgggatgccccatccactgtatggctatgattctactatcgtcttatttctatttcctccaaaacactgctgacatatacctcagttggatgtttggccttctggtcctctataagtccctaagcatgctcctgggccttcagagcttgactccagcggaagtctctgcagtctgtgaagaaaagaagttaaatgttgcccacgggctggcctggtcatactacattgggtacttgcggttgatcttaccagggctccaggcccggatccgaatgttcaatcagctacataacaacatgctcagtggtgcagggagccgaagactgtacatcctctttccattggactgtggggtgcctgacaacctgagtgtagttgaccccaacattcgattccgagatatgctgccccagcaaaacatcgaccgtgctggcatcaagaatcgggtttattccaacagcgtctacgagattctggagaacggacagccagcaggcgtctgtatcctggagtacgccacccccttgcagaccctgtttgccatgtcacaggatgccaaagctggcttcagtcgggaggatcggcttgagcaggctaaactcttctgccggacacttgaggaaatcctggaagatgtccccgagtctcgaaataactgccgcctcattgtctaccaagaacccacagacggaaacagtttctcactgtctcaggaggtgctccggcacattcgtcaggaagaaaaggaggaggttaccatgaatgcccccatgacctcagtggcacctcctccctccgtactgtcccaagagccaagactcctcatcagtggtatggatcagcctctcccactccgcactgacctcatctga

SEQ ID NO: 21 - protein, 243 aa, Homo sapiens
MGSSHHHHHHSSGSGLNDIFEAQKIEWHEGGSENLYFQGLAPAEISAVCEKGNFNVAHGLAWSYYIGYLRLILPELQARIRTYNQHYNNLLRGAVSQRLYILLPLDCGVPDNLSMADPNIRFLDKLPQQTGDRAGIKDRVYSNSIYELLENGQRAGTCVLEYATPLQTLFAMSQYSQAGFSREDRLEQAKLFCRTLEDILADAPESQNNCRLIAYQEPADDSSFSLSQEVLRHLRQEEKEEVT

SEQ ID NO: 22 - protein, 243 aa, Homo sapiens
MGSSHHHHHHSSGSGLNDIFEAQKIEWHEGGSENLYFQGLAPAEISAVCEKGNFNVAHGLAWSYYIGYLRLILPELQARIRTYNQHYNNLLRGAVSQRLYILLPLDCGVPDNLSMADPNIRFLDKLPQQTGDHAGIKDRVYSNSIYELLENGQRAGTCVLEYATPLQTLFAMSQYSQAGFSREDRLEQAKLFCRTLEDILADAPESQNNCRLIAYQEPADDSSFSLSQEVLRHLRQEEKEEVT

SEQ ID NO: 23 - protein, 243 aa, Homo sapiens
MGSSHHHHHHSSGSGLNDIFEAQKIEWHEGGSENLYFQGLAPAEISAVCEKGNFNVAHGLAWSYYIGYLRLILPELQARIRTYNQHYNNLLRGAVSQRLYILLPLDCGVPDNLSMADPNIRFLDKLPQQTADRAGIKDRVYSNSIYELLENGQRAGTCVLEYATPLQTLFAMSQYSQAGFSREDRLEQAKLFCQTLEDILADAPESQNNCRLIAYQEPADDSSFSLSQEVLRHLRQEEKEEVT

SEQ ID NO: 24 - protein, 243 aa, Homo sapiens
MGSSHHHHHHSSGSGLNDIFEAQKIEWHEGGSENLYFQGLTPAEVSAVCEEKKLNVAHGLAWSYYIGYLRLILPGLQARIRMFNQLHNNMLSGAGSRRLYILFPLDCGVPDNLSVVDPNIRFRDMLPQQNIDRAGIKNRVYSNSVYEILENGQPAGVCILEYATPLQTLFAMSQDAKAGFSREDRLEQAKLFCRTLEEILEDVPESRNNCRLIVYQEPTDGNSFSLSQEVLRHIRQEEKEEVT

SEQ ID NO: 25 - DNA, 27 bp, Artificial Sequence
  primer
cgtgctggcatcaaggatcgggtttac

SEQ ID NO: 26 - DNA, 27 bp, Artificial Sequence
  primer
gtcaccggtctgctggggcagtttatc

SEQ ID NO: 27 - DNA, 33 bp, Artificial Sequence
  primer
gctgaccgtgctggcatcaaggatcgggtttac

SEQ ID NO: 28 - DNA, 25 bp, Artificial Sequence
  primer
ggtctgctggggcagtttatccagg

SEQ ID NO: 29 - DNA, 24 bp, Artificial Sequence
  primer
caccacatccactccaggtaccgg

SEQ ID NO: 30 - DNA, 24 bp, Artificial Sequence
  primer
cagctcctcagccaggctgcagac

SEQ ID NO: 31 - DNA, 25 bp, Artificial Sequence
  primer
cagacacttgaggacatcctggcag

SEQ ID NO: 32 - DNA, 23 bp, Artificial Sequence
  primer
gcagaagagtttggcctgctcaa

SEQ ID NO: 33 - DNA, 39 bp, Artificial Sequence
  primer
acctgtattttcagggcctggccccagctgagatctctg

SEQ ID NO: 34 - DNA, 44 bp, Artificial Sequence
  primer
cagaattcgcaagcttttaagtaacctcttccttttcctcctgc

SEQ ID NO: 35 - protein, 15 aa, Homo sapiens
RASKSVSTSGYSFMH

SEQ ID NO: 36 - protein, 7 aa, Homo sapiens
LASNLES

SEQ ID NO: 37 - protein, 9 aa, Homo sapiens
QHSREVPWT

SEQ ID NO: 38 - protein, 10 aa, Homo sapiens
GYTFTNYGMN

SEQ ID NO: 39 - protein, 17 aa, Homo sapiens
WINTYTGEPTYADAFKG

SEQ ID NO: 40 - protein, 9 aa, Homo sapiens
DYGDYGMDY

SEQ ID NO: 41 - protein, 11 aa, Homo sapiens
RASQSVSSYLA

SEQ ID NO: 42 - protein, 7 aa, Homo sapiens
DASNRAT

SEQ ID NO: 43 - protein, 9 aa, Homo sapiens
QQRTNWPLT

SEQ ID NO: 44 - protein, 5 aa, Homo sapiens
SYIMH

SEQ ID NO: 45 - protein, 17 aa, Homo sapiens
VISYDGRNKYYADSVKG

SEQ ID NO: 46 - protein, 9 aa, Homo sapiens
DTDGYDFDY

SEQ ID NO: 47 - protein, 11 aa, Homo sapiens
KASQDVSTAVA

SEQ ID NO: 48 - protein, 7 aa, Homo sapiens
SASYRYT

SEQ ID NO: 49 - protein, 9 aa, Homo sapiens
QQHYITPLT

SEQ ID NO: 50 - protein, 5 aa, Homo sapiens
TAGMQ

SEQ ID NO: 51 - protein, 17 aa, Homo sapiens
WINTHSGVPKYAEDFKG

SEQ ID NO: 52 - protein, 12 aa, Homo sapiens
SGFGSSYWYFDV

SEQ ID NO: 53 - protein, 11 aa, Homo sapiens
KASQDVSTAVA

SEQ ID NO: 54 - protein, 7 aa, Homo sapiens
SASYRYT

SEQ ID NO: 55 - protein, 9 aa, Homo sapiens
QQHYITPLT

SEQ ID NO: 56 - protein, 5 aa, Homo sapiens
TAGMQ

SEQ ID NO: 57 - protein, 17 aa, Homo sapiens
WINTHSGVPKYAEDFKG

SEQ ID NO: 58 - protein, 12 aa, Homo sapiens
SGFGSSYWYFDV

SEQ ID NO: 59 - protein, 11 aa, Homo sapiens
QASQDISNYLN

SEQ ID NO: 60 - protein, 7 aa, Homo sapiens
DASNLET

SEQ ID NO: 61 - protein, 9 aa, Homo sapiens
QHFDHLPLA

SEQ ID NO: 62 - protein, 7 aa, Homo sapiens
SGDYYWT

SEQ ID NO: 63 - protein, 17 aa, Homo sapiens
GHIYYSGNTNYNPSLKS

SEQ ID NO: 64 - protein, 9 aa, Homo sapiens
DRVTGAFDI

SEQ ID NO: 65 - protein, 11 aa, Homo sapiens
HSSQDINSNIG

SEQ ID NO: 66 - protein, 7 aa, Homo sapiens
HGTNLDD

SEQ ID NO: 67 - protein, 9 aa, Homo sapiens
VQYAQFPWT

SEQ ID NO: 68 - protein, 11 aa, Homo sapiens
GYSITSDFAWN

SEQ ID NO: 69 - protein, 16 aa, Homo sapiens
GYISYSGNTRYNPSLK

SEQ ID NO: 70 - protein, 9 aa, Homo sapiens
VTAGRGFPY